European Patent Application EP 4 403 570 A2, published July 24, 2024. Title: Anti-IL-33 Antibodies and Uses Thereof. Applicant: Regeneron Pharmaceuticals, Inc. The sequence listing filed with the application follows.

SEQUENCE LISTING (323 sequences)

SEQ ID NO: 1 - DNA, 366 bp, synthetic construct
  misc_feature 1..366: note = Synthetic
  source 1..366: mol_type = other DNA
caggtgcagctggtggagtctgggggaggcgtggtccagcctgggaggtccctgagactctcctgtgcagcgtctggattcaccttcagtagttatggcatgcattgggtccgccaggctccaggcaaggggctggagtgggtggcagttatatggtatgatggaagaaataaatactatacagactccgtgaagggccgattcaccatctccagagacaattccaagaacacgctgtatctgcaaatggacagcctgagagccgaggacacggctgtgtattactgtgcgagagagaggtatatcagcagctattatggggggttcgacccctggggccagggagccctggtcaccgtctcctca

SEQ ID NO: 2 - protein, 122 aa, synthetic construct
  REGION 1..122: note = Synthetic
QVQLVESGGGVVQPGRSLRLSCAASGFTFSSYGMHWVRQAPGKGLEWVAVIWYDGRNKYYTDSVKGRFTISRDNSKNTLYLQMDSLRAEDTAVYYCARERYISSYYGGFDPWGQGALVTVSS

SEQ ID NO: 3 - DNA, 24 bp, synthetic construct
  misc_feature 1..24: note = Synthetic
  source 1..24: mol_type = other DNA
ggattcaccttcagtagttatggc

SEQ ID NO: 4 - protein, 8 aa, synthetic construct
  REGION 1..8: note = Synthetic
GFTFSSYG

SEQ ID NO: 5 - DNA, 24 bp, synthetic construct
  misc_feature 1..24: note = Synthetic
  source 1..24: mol_type = other DNA
atatggtatgatggaagaaataaa

SEQ ID NO: 6 - protein, 8 aa, synthetic construct
  REGION 1..8: note = Synthetic
IWYDGRNK

SEQ ID NO: 7 - DNA, 45 bp, synthetic construct
  misc_feature 1..45: note = Synthetic
  source 1..45: mol_type = other DNA
gcgagagagaggtatatcagcagctattatggggggttcgacccc

SEQ ID NO: 8 - protein, 15 aa, synthetic construct
  REGION 1..15: note = Synthetic
ARERYISSYYGGFDP

SEQ ID NO: 9 - DNA, 321 bp, synthetic construct
  misc_feature 1..321: note = Synthetic
  source 1..321: mol_type = other DNA
gacatccagatgacccagtctccatcctccgtgtctgcatctgtaggagacagagtcaccatcacttgtcgggcgagtcagggtattagtagttggttagcctggtatcagcagaaaccagggaaagcccctaaggtcctgatctatgctgcatccagtttgcaaagtggggtcccatcaaggttcagcggcagtggatctgggacagatttcactctcaccatcagcagcctgcagcctgaagattttgcaacttactattgtcaacaggctaacagtttcccattcactttcggccctgggaccaaactggatatcaag

SEQ ID NO: 10 - protein, 107 aa, synthetic construct
  REGION 1..107: note = Synthetic
DIQMTQSPSSVSASVGDRVTITCRASQGISSWLAWYQQKPGKAPKVLIYAASSLQSGVPSRFSGSGSGTDFTLTISSLQPEDFATYYCQQANSFPFTFGPGTKLDIK

SEQ ID NO: 11 - DNA, 18 bp, synthetic construct
  misc_feature 1..18: note = Synthetic
  source 1..18: mol_type = other DNA
cagggtattagtagttgg

SEQ ID NO: 12 - protein, 6 aa, synthetic construct
  REGION 1..6: note = Synthetic
QGISSW

SEQ ID NO: 13-14 - skipped (2 entries)

SEQ ID NO: 15 - DNA, 27 bp, synthetic construct
  misc_feature 1..27: note = Synthetic
  source 1..27: mol_type = other DNA
caacaggctaacagtttcccattcact

SEQ ID NO: 16 - protein, 9 aa, synthetic construct
  REGION 1..9: note = Synthetic
QQANSFPFT

SEQ ID NO: 17 - DNA, 357 bp, synthetic construct
  misc_feature 1..357: note = Synthetic
  source 1..357: mol_type = other DNA
gaggtgcagctgttggagtctgggggagacttggtacagcctggggggtccctgagactctcctgtgcagcctctggattcaccttcagcagctatgccatgagctgggtccgccaggctccagggaaggggctggagtgggtctcagttattagtggtagtggaagtagcacagactacgcagactccgtgaagggccggttcaccatttccagagacaattccagggacacgctgcatctgcaaatgaacagcctgagagccgaggacacggccgtatattactgtgcgaaaacgttctactacttctacggtttggacgtctggggccaagggaccacggtcaccgtctcctca

SEQ ID NO: 18 - protein, 119 aa, synthetic construct
  REGION 1..119: note = Synthetic
EVQLLESGGDLVQPGGSLRLSCAASGFTFSSYAMSWVRQAPGKGLEWVSVISGSGSSTDYADSVKGRFTISRDNSRDTLHLQMNSLRAEDTAVYYCAKTFYYFYGLDVWGQGTTVTVSS

SEQ ID NO: 19 - DNA, 24 bp, synthetic construct
  misc_feature 1..24: note = Synthetic
  source 1..24: mol_type = other DNA
ggattcaccttcagcagctatgcc

SEQ ID NO: 20 - protein, 8 aa, synthetic construct
  REGION 1..8: note = Synthetic
GFTFSSYA

SEQ ID NO: 21 - DNA, 24 bp, synthetic construct
  misc_feature 1..24: note = Synthetic
  source 1..24: mol_type = other DNA
attagtggtagtggaagtagcaca

SEQ ID NO: 22 - protein, 8 aa, synthetic construct
  REGION 1..8: note = Synthetic
ISGSGSST

SEQ ID NO: 23 - DNA, 36 bp, synthetic construct
  misc_feature 1..36: note = Synthetic
  source 1..36: mol_type = other DNA
gcgaaaacgttctactacttctacggtttggacgtc

SEQ ID NO: 24 - protein, 12 aa, synthetic construct
  REGION 1..12: note = Synthetic
AKTFYYFYGLDV

SEQ ID NO: 25 - DNA, 321 bp, synthetic construct
  misc_feature 1..321: note = Synthetic
  source 1..321: mol_type = other DNA
gacatccagatgacccagtctccatcctccctgtctgcatctttaagagacagagtcaccatcacttgccgggcgagtcagggcattagcaattatttagcctggtatcagcagaaaccagggaaagttcctaaggtcctaatctatgctgcatccactttgcaatcaggggtcccatctcggttcagtggcagtggatctgggacagttttcactctcaccatcagcagcctgcagactgaagatgttgcaacttattactgtcaaaagtatagcagtgccccattcactttcggccctgggaccaaagtggatatcaaa

SEQ ID NO: 26 - protein, 107 aa, synthetic construct
  REGION 1..107: note = Synthetic
DIQMTQSPSSLSASLRDRVTITCRASQGISNYLAWYQQKPGKVPKVLIYAASTLQSGVPSRFSGSGSGTVFTLTISSLQTEDVATYYCQKYSSAPFTFGPGTKVDIK

SEQ ID NO: 27 - DNA, 18 bp, synthetic construct
  misc_feature 1..18: note = Synthetic
  source 1..18: mol_type = other DNA
cagggcattagcaattat

SEQ ID NO: 28 - protein, 6 aa, synthetic construct
  REGION 1..6: note = Synthetic
QGISNY

SEQ ID NO: 29-30 - skipped (2 entries)

SEQ ID NO: 31 - DNA, 27 bp, synthetic construct
  misc_feature 1..27: note = Synthetic
  source 1..27: mol_type = other DNA
caaaagtatagcagtgccccattcact

SEQ ID NO: 32 - protein, 9 aa, synthetic construct
  REGION 1..9: note = Synthetic
QKYSSAPFT

SEQ ID NO: 33 - DNA, 351 bp, synthetic construct
  misc_feature 1..351: note = Synthetic
  source 1..351: mol_type = other DNA
caggtgcttctggtacagtctggggctgaggtgaagaagcctggggccacagtgaaggtctcctgcaaggcttctggatccactttcaccggctactatatgcactgggtgcgacaggcccctggacaagggcttgagtggatgggatggatcaaccctaacaatggtggcacaaactatgcacagaagtttcagggcagggtcaccatgaccagggacacgtccatcagcacagcctacatggaattgagcaggctgagatctgacgacacggccgtatattactgtgcgagagagttgcggtataactggaagtcctggggccagggaaccctggtcaccgtctcctca

SEQ ID NO: 34 - protein, 117 aa, synthetic construct
  REGION 1..117: note = Synthetic
QVLLVQSGAEVKKPGATVKVSCKASGSTFTGYYMHWVRQAPGQGLEWMGWINPNNGGTNYAQKFQGRVTMTRDTSISTAYMELSRLRSDDTAVYYCARELRYNWKSWGQGTLVTVSS

SEQ ID NO: 35 - DNA, 24 bp, synthetic construct
  misc_feature 1..24: note = Synthetic
  source 1..24: mol_type = other DNA
ggatccactttcaccggctactat

SEQ ID NO: 36 - protein, 8 aa, synthetic construct
  REGION 1..8: note = Synthetic
GSTFTGYY

SEQ ID NO: 37 - DNA, 24 bp, synthetic construct
  misc_feature 1..24: note = Synthetic
  source 1..24: mol_type = other DNA
atcaaccctaacaatggtggcaca

SEQ ID NO: 38 - protein, 8 aa, synthetic construct
  REGION 1..8: note = Synthetic
INPNNGGT

SEQ ID NO: 39 - DNA, 30 bp, synthetic construct
  misc_feature 1..30: note = Synthetic
  source 1..30: mol_type = other DNA
gcgagagagttgcggtataactggaagtcc

SEQ ID NO: 40 - protein, 10 aa, synthetic construct
  REGION 1..10: note = Synthetic
ARELRYNWKS

SEQ ID NO: 41 - DNA, 324 bp, synthetic construct
  misc_feature 1..324: note = Synthetic
  source 1..324: mol_type = other DNA
gaaattgtgttgacgcagtctccaggcaccctgtctttgtctccaggggaaagagtcaccctctcctgcagggccagtcagagtgttggcaggccctacttagcctggtaccaacagatacctggccaggctcccaggctcctcatctatggtgcatccagcagggccactgacatcccagacaggttcagtggcaatgggtctgggacagacttcactctcaccatcagtagactggagcctgaagattttgcagtgtattactgtcagcagtatgataattccccttatacttttggccaggggaccaggctggagatcaaa

SEQ ID NO: 42 - protein, 108 aa, synthetic construct
  REGION 1..108: note = Synthetic
EIVLTQSPGTLSLSPGERVTLSCRASQSVGRPYLAWYQQIPGQAPRLLIYGASSRATDIPDRFSGNGSGTDFTLTISRLEPEDFAVYYCQQYDNSPYTFGQGTRLEIK

SEQ ID NO: 43 - DNA, 21 bp, synthetic construct
  misc_feature 1..21: note = Synthetic
  source 1..21: mol_type = other DNA
cagagtgttggcaggccctac

SEQ ID NO: 44 - protein, 7 aa, synthetic construct
  REGION 1..7: note = Synthetic
QSVGRPY

SEQ ID NO: 45-46 - skipped (2 entries)

SEQ ID NO: 47 - DNA, 27 bp, synthetic construct
  misc_feature 1..27: note = Synthetic
  source 1..27: mol_type = other DNA
cagcagtatgataattccccttatact

SEQ ID NO: 48 - protein, 9 aa, synthetic construct
  REGION 1..9: note = Synthetic
QQYDNSPYT

SEQ ID NO: 49 - DNA, 366 bp, synthetic construct
  misc_feature 1..366: note = Synthetic
  source 1..366: mol_type = other DNA
gaggtgcagctggtggagtctgggggaggcttggtacaacctggggggtccctgagactctcctgtgcagcctctggattcacctttagaagctttgccatgagctgggtccgccaggctccagggaaggggctggaattggtctcagatctcaggactagtggtggtagtacatactacgcagactccgtgaagggccggctcaccatctccagagacaattccaagaacacgctgtatctgcaaatgaacagcctgagagccgaggacacggccgtatattactgtgcgaaaagccactatagcaccagctggttcgggggctttgactactggggccagggaaccctggtcactgtctcctca

SEQ ID NO: 50 - protein, 122 aa, synthetic construct
  REGION 1..122: note = Synthetic
EVQLVESGGGLVQPGGSLRLSCAASGFTFRSFAMSWVRQAPGKGLELVSDLRTSGGSTYYADSVKGRLTISRDNSKNTLYLQMNSLRAEDTAVYYCAKSHYSTSWFGGFDYWGQGTLVTVSS

SEQ ID NO: 51 - DNA, 24 bp, synthetic construct
  misc_feature 1..24: note = Synthetic
  source 1..24: mol_type = other DNA
ggattcacctttagaagctttgcc

SEQ ID NO: 52 - protein, 8 aa, synthetic construct
  REGION 1..8: note = Synthetic
GFTFRSFA

SEQ ID NO: 53 - DNA, 24 bp, synthetic construct
  misc_feature 1..24: note = Synthetic
  source 1..24: mol_type = other DNA
ctcaggactagtggtggtagtaca

SEQ ID NO: 54 - protein, 8 aa, synthetic construct
  REGION 1..8: note = Synthetic
LRTSGGST

SEQ ID NO: 55 - DNA, 45 bp, synthetic construct
  misc_feature 1..45: note = Synthetic
  source 1..45: mol_type = other DNA
gcgaaaagccactatagcaccagctggttcgggggctttgactac

SEQ ID NO: 56 - protein, 15 aa, synthetic construct
  REGION 1..15: note = Synthetic
AKSHYSTSWFGGFDY

SEQ ID NO: 57 - DNA, 321 bp, synthetic construct
  misc_feature 1..321: note = Synthetic
  source 1..321: mol_type = other DNA
gacatccagatgacccagtctccatcttccgtgtctgcttctgtaggagacagagtcaccatcacttgtcgggcgagtcagggttttagcagctggttagcctggtatcagcagaaaccagggaaagcccctaagctcctgatctatgctgcatccagtttgcaaagtggggtcccatcaaggttcagcggcagtggatctgggacagatttcactctcaccatcaccaacctgcagcctgaagattttgcaacttactattgtcaacaggctaacagtttccctctcactttcggcggagggaccaaggtggagatcaaa

SEQ ID NO: 58 - protein, 107 aa, synthetic construct
  REGION 1..107: note = Synthetic
DIQMTQSPSSVSASVGDRVTITCRASQGFSSWLAWYQQKPGKAPKLLIYAASSLQSGVPSRFSGSGSGTDFTLTITNLQPEDFATYYCQQANSFPLTFGGGTKVEIK

SEQ ID NO: 59 - DNA, 18 bp, synthetic construct
  misc_feature 1..18: note = Synthetic
  source 1..18: mol_type = other DNA
cagggttttagcagctgg

SEQ ID NO: 60 - protein, 6 aa, synthetic construct
  REGION 1..6: note = Synthetic
QGFSSW

SEQ ID NO: 61-62 - skipped (2 entries)

SEQ ID NO: 63 - DNA, 27 bp, synthetic construct
  misc_feature 1..27: note = Synthetic
  source 1..27: mol_type = other DNA
caacaggctaacagtttccctctcact

SEQ ID NO: 64 - protein, 9 aa, synthetic construct
  REGION 1..9: note = Synthetic
QQANSFPLT

SEQ ID NO: 65 - DNA, 366 bp, synthetic construct
  misc_feature 1..366: note = Synthetic
  source 1..366: mol_type = other DNA
gaggtgcagctggtggagtctgggggaggcttggtacagcctggggggtccctgagactctcctgtgcagcctctggattcacgtttagcagctatgtcatgagctgggtccgccaggctccagggaaggggctggagtgggtctcaagtattagtggtaatggtggtagcacaaactacgcagactccgtgaagggccggttcaccatctccagagacaattccaagaacacgctgtttctggaaatgaacagcctgagagccgaggacacggccgtatattactgtgcgaaatcactgggaactaccacgacttttttggggtttgactattggggccagggaaccctggtcaccgtctcctca

SEQ ID NO: 66 - protein, 122 aa, synthetic construct
  REGION 1..122: note = Synthetic
EVQLVESGGGLVQPGGSLRLSCAASGFTFSSYVMSWVRQAPGKGLEWVSSISGNGGSTNYADSVKGRFTISRDNSKNTLFLEMNSLRAEDTAVYYCAKSLGTTTTFLGFDYWGQGTLVTVSS

SEQ ID NO: 67 - DNA, 24 bp, synthetic construct
  misc_feature 1..24: note = Synthetic
  source 1..24: mol_type = other DNA
ggattcacgtttagcagctatgtc

SEQ ID NO: 68 - protein, 8 aa, synthetic construct
  REGION 1..8: note = Synthetic
GFTFSSYV

SEQ ID NO: 69 - DNA, 24 bp, synthetic construct
  misc_feature 1..24: note = Synthetic
  source 1..24: mol_type = other DNA
attagtggtaatggtggtagcaca

SEQ ID NO: 70 - protein, 8 aa, synthetic construct
  REGION 1..8: note = Synthetic
ISGNGGST

SEQ ID NO: 71 - DNA, 45 bp, synthetic construct
  misc_feature 1..45: note = Synthetic
  source 1..45: mol_type = other DNA
gcgaaatcactgggaactaccacgacttttttggggtttgactat

SEQ ID NO: 72 - protein, 15 aa, synthetic construct
  REGION 1..15: note = Synthetic
AKSLGTTTTFLGFDY

SEQ ID NO: 73 - DNA, 321 bp, synthetic construct
  misc_feature 1..321: note = Synthetic
  source 1..321: mol_type = other DNA
gacatccagatgacccagtctccatcttccgtgtctgcatctgtaggagacagagtcaccatcacttgtcgggcgagtcagggtattagcagctggttagcctggtatcagcagaaaccagggaaagcccctaaactcctgatctatgctgcatccagtttgcaaagtggggtcccatcaaggttcagcggcagtggatctgggacatatttcactctcaccatcagcagcctgcagcctgaagattttgcaacttactattgtcaacaggctaacagtttccctctcactttcggcggagggaccaaggtggagatcaaa

SEQ ID NO: 74 - protein, 107 aa, synthetic construct
  REGION 1..107: note = Synthetic
DIQMTQSPSSVSASVGDRVTITCRASQGISSWLAWYQQKPGKAPKLLIYAASSLQSGVPSRFSGSGSGTYFTLTISSLQPEDFATYYCQQANSFPLTFGGGTKVEIK

SEQ ID NO: 75 - DNA, 18 bp, synthetic construct
  misc_feature 1..18: note = Synthetic
  source 1..18: mol_type = other DNA
cagggtattagcagctgg

SEQ ID NO: 76 - protein, 6 aa, synthetic construct
  REGION 1..6: note = Synthetic
QGISSW

SEQ ID NO: 77-78 - skipped (2 entries)

SEQ ID NO: 79 - DNA, 27 bp, synthetic construct
  misc_feature 1..27: note = Synthetic
  source 1..27: mol_type = other DNA
caacaggctaacagtttccctctcact

SEQ ID NO: 80 - protein, 9 aa, synthetic construct
  REGION 1..9: note = Synthetic
QQANSFPLT

SEQ ID NO: 81 - DNA, 363 bp, synthetic construct
  misc_feature 1..363: note = Synthetic
  source 1..363: mol_type = other DNA
caggtgcagctgcaggagtcgggcccaggactggtgaagccttcggagaccctgtccctcacctgcactgtctctggtggctccatcagtagttattactggagctggatccggcagcccccagggaagggactggagttgattgggtatatttattacagtgggagcaccaattataacccctccctcaagagtcgagtcaccatatctgtagacacgtccaagaaccacttctccctgaagctgagctctgtgaccgctgcggacacggccgtatattactgtgcgagatcccagtataccagtagttggtacggttcttttgatatctggggccaagggacaatggtcaccgtctcttca

SEQ ID NO: 82 - protein, 121 aa, synthetic construct
  REGION 1..121: note = Synthetic
QVQLQESGPGLVKPSETLSLTCTVSGGSISSYYWSWIRQPPGKGLELIGYIYYSGSTNYNPSLKSRVTISVDTSKNHFSLKLSSVTAADTAVYYCARSQYTSSWYGSFDIWGQGTMVTVSS

SEQ ID NO: 83 - DNA, 24 bp, synthetic construct
  misc_feature 1..24: note = Synthetic
  source 1..24: mol_type = other DNA
ggtggctccatcagtagttattac

SEQ ID NO: 84 - protein, 8 aa, synthetic construct
  REGION 1..8: note = Synthetic
GGSISSYY

SEQ ID NO: 85 - DNA, 21 bp, synthetic construct
  misc_feature 1..21: note = Synthetic
  source 1..21: mol_type = other DNA
atttattacagtgggagcacc

SEQ ID NO: 86 - protein, 7 aa, synthetic construct
  REGION 1..7: note = Synthetic
IYYSGST

SEQ ID NO: 87 - DNA, 45 bp, synthetic construct
  misc_feature 1..45: note = Synthetic
  source 1..45: mol_type = other DNA
gcgagatcccagtataccagtagttggtacggttcttttgatatc

SEQ ID NO: 88 - protein, 15 aa, synthetic construct
  REGION 1..15: note = Synthetic
ARSQYTSSWYGSFDI

SEQ ID NO: 89 - DNA, 321 bp, synthetic construct
  misc_feature 1..321: note = Synthetic
  source 1..321: mol_type = other DNA
gacatccagatgacccagtctccatcttccgtgtctgcatctgtaggagacagagtcaccatcacttgtcgggcgagtcagggtattagcacctggttagcctggtttcagcagaaaccagggaaagcccctaagctcctgatctatgctgcatccactttacaaggtggggtcccatcaaggttcagcggcagtggatctgggccagaattcactctcaccatcagcagcctgcagcctgaagattttgcaacttactattgtcaacaggctaacagtttcccgtggacgttcggccaagggaccaaggtggaaatcaaa

SEQ ID NO: 90 - protein, 107 aa, synthetic construct
  REGION 1..107: note = Synthetic
DIQMTQSPSSVSASVGDRVTITCRASQGISTWLAWFQQKPGKAPKLLIYAASTLQGGVPSRFSGSGSGPEFTLTISSLQPEDFATYYCQQANSFPWTFGQGTKVEIK

SEQ ID NO: 91 - DNA, 18 bp, synthetic construct
  misc_feature 1..18: note = Synthetic
  source 1..18: mol_type = other DNA
cagggtattagcacctgg

SEQ ID NO: 92 - protein, 6 aa, synthetic construct
  REGION 1..6: note = Synthetic
QGISTW

SEQ ID NO: 93-94 - skipped (2 entries)

SEQ ID NO: 95 - DNA, 27 bp, synthetic construct
  misc_feature 1..27: note = Synthetic
  source 1..27: mol_type = other DNA
caacaggctaacagtttcccgtggacg

SEQ ID NO: 96 - protein, 9 aa, synthetic construct
  REGION 1..9: note = Synthetic
QQANSFPWT

SEQ ID NO: 97 - DNA, 366 bp, synthetic construct
  misc_feature 1..366: note = Synthetic
  source 1..366: mol_type = other DNA
caggttcagctggtgcagtctggagctgaggtgaagaagcctggggcctcagtgaaggtctcctgcaaggcctctggttacacctttaacagctatggtatcagctgggtgcgacaggcccctggacaagggcttgagtggatgggatggatcagctcccacaatggtaacagtcactatgtacagaagttccagggcagagtctccatgaccacagacacatccacgagtacagcctacatggaactgaggagccttagatctgacgacacggccgtgtattactgtgcgagacactcgtataccaccagctggtacgggggttttgactattggggccagggaaccctggtcaccgtctcctca

SEQ ID NO: 98 - protein, 122 aa, synthetic construct
  REGION 1..122: note = Synthetic
QVQLVQSGAEVKKPGASVKVSCKASGYTFNSYGISWVRQAPGQGLEWMGWISSHNGNSHYVQKFQGRVSMTTDTSTSTAYMELRSLRSDDTAVYYCARHSYTTSWYGGFDYWGQGTLVTVSS

SEQ ID NO: 99 - DNA, 24 bp, synthetic construct
  misc_feature 1..24: note = Synthetic
  source 1..24: mol_type = other DNA
ggttacacctttaacagctatggt

SEQ ID NO: 100 - protein, 8 aa, synthetic construct
  REGION 1..8: note = Synthetic
GYTFNSYG

SEQ ID NO: 101 - DNA, 24 bp, synthetic construct
  misc_feature 1..24: note = Synthetic
  source 1..24: mol_type = other DNA
atcagctcccacaatggtaacagt

SEQ ID NO: 102 - protein, 8 aa, synthetic construct
  REGION 1..8: note = Synthetic
ISSHNGNS

SEQ ID NO: 103 - DNA, 45 bp, synthetic construct
  misc_feature 1..45: note = Synthetic
  source 1..45: mol_type = other DNA
gcgagacactcgtataccaccagctggtacgggggttttgactat

SEQ ID NO: 104 - protein, 15 aa, synthetic construct
  REGION 1..15: note = Synthetic
ARHSYTTSWYGGFDY

SEQ ID NO: 105 - DNA, 321 bp, synthetic construct
  misc_feature 1..321: note = Synthetic
  source 1..321: mol_type = other DNA
gacatccagatgacccagtctccatcttccgtgtctgcatctgtaggagacagagtcaccatcacttgtcgggcgagtcagggttttagcagctggttagcctggtatcagcagaaaccagggaaagcccctcagctcctgatctatgctgcatccagtttgcaaagtggggtcccatcaaggttcagcggcagtggatctgggtcagatttcactctcaccatcagcagcctgcagcctgaagattttgcaacttactattgtcaacaggctaacagtttccctctcactttcggcggagggaccaaggtggagatcaaa

SEQ ID NO: 106 - protein, 107 aa, synthetic construct
  REGION 1..107: note = Synthetic
DIQMTQSPSSVSASVGDRVTITCRASQGFSSWLAWYQQKPGKAPQLLIYAASSLQSGVPSRFSGSGSGSDFTLTISSLQPEDFATYYCQQANSFPLTFGGGTKVEIK

SEQ ID NO: 107 - DNA, 18 bp, synthetic construct
  misc_feature 1..18: note = Synthetic
  source 1..18: mol_type = other DNA
cagggttttagcagctgg

SEQ ID NO: 108 - protein, 6 aa, synthetic construct
  REGION 1..6: note = Synthetic
QGFSSW

SEQ ID NO: 109-110 - skipped (2 entries)

SEQ ID NO: 111 - DNA, 27 bp, synthetic construct
  misc_feature 1..27: note = Synthetic
  source 1..27: mol_type = other DNA
caacaggctaacagtttccctctcact

SEQ ID NO: 112 - protein, 9 aa, synthetic construct
  REGION 1..9: note = Synthetic
QQANSFPLT

SEQ ID NO: 113 - DNA, 366 bp, synthetic construct
  misc_feature 1..366: note = Synthetic
  source 1..366: mol_type = other DNA
gaggtgcagctggtggagtccgggggaggcttggttcagccgggggggtccctgagactctcctgtgcagcctctggaatcaccttgagcagctatggcatgagctgggtccgccaggctccagggaagggactggagtgggtcgcatccatttttggtagtggtggtggcccatactacgcagactccgtgaagggccggttcaccatgtccagagacaattccaagaacacgctgtatttgcaaatgaacagcctgagagccgaggacacggccgtatattattgtgcgaaagatcgatacagtgggagctactacggaggttttgactactggggccggggaaccctggtcaccgtctcctca

SEQ ID NO: 114 - protein, 122 aa, synthetic construct
  REGION 1..122: note = Synthetic
EVQLVESGGGLVQPGGSLRLSCAASGITLSSYGMSWVRQAPGKGLEWVASIFGSGGGPYYADSVKGRFTMSRDNSKNTLYLQMNSLRAEDTAVYYCAKDRYSGSYYGGFDYWGRGTLVTVSS

SEQ ID NO: 115 - DNA, 24 bp, synthetic construct
  misc_feature 1..24: note = Synthetic
  source 1..24: mol_type = other DNA
ggaatcaccttgagcagctatggc

SEQ ID NO: 116 - protein, 8 aa, synthetic construct
  REGION 1..8: note = Synthetic
GITLSSYG

SEQ ID NO: 117 - DNA, 24 bp, synthetic construct
  misc_feature 1..24: note = Synthetic
  source 1..24: mol_type = other DNA
atttttggtagtggtggtggccca

SEQ ID NO: 118 - protein, 8 aa, synthetic construct
  REGION 1..8: note = Synthetic
IFGSGGGP

SEQ ID NO: 119 - DNA, 45 bp, synthetic construct
  misc_feature 1..45: note = Synthetic
  source 1..45: mol_type = other DNA
gcgaaagatcgatacagtgggagctactacggaggttttgactac

SEQ ID NO: 120 - protein, 15 aa, synthetic construct
  REGION 1..15: note = Synthetic
AKDRYSGSYYGGFDY

SEQ ID NO: 121 - DNA, 321 bp, synthetic construct
  misc_feature 1..321: note = Synthetic
  source 1..321: mol_type = other DNA
gacatccagatgacccagtctccatcttccgtgtctgcatctgtaggagacagagtcaccatcacttgtcgggcgagtcagggtattaccagctggttagcctggtatcagcagaaaccagggaaagcccctacactcctgatctatgctgcatccagtttgcaaactggggtcccatcaaggttcagcggcagtggatctgggacagatttcactctcaccatcagcagcctgcagcctgaacattttgcaacttactattgtcaacaggctaacagtttccctcctactttcggcggagggaccaaggtggagatcaaa

SEQ ID NO: 122 - protein, 107 aa, synthetic construct
  REGION 1..107: note = Synthetic
DIQMTQSPSSVSASVGDRVTITCRASQGITSWLAWYQQKPGKAPTLLIYAASSLQTGVPSRFSGSGSGTDFTLTISSLQPEHFATYYCQQANSFPPTFGGGTKVEIK

SEQ ID NO: 123 - DNA, 18 bp, synthetic construct
  misc_feature 1..18: note = Synthetic
  source 1..18: mol_type = other DNA
cagggtattaccagctgg

SEQ ID NO: 124 - protein, 6 aa, synthetic construct
  REGION 1..6: note = Synthetic
QGITSW

SEQ ID NO: 125-126 - skipped (2 entries)

SEQ ID NO: 127 - DNA, 27 bp, synthetic construct
  misc_feature 1..27: note = Synthetic
  source 1..27: mol_type = other DNA
caacaggctaacagtttccctcctact

SEQ ID NO: 128 - protein, 9 aa, synthetic construct
  REGION 1..9: note = Synthetic
QQANSFPPT

SEQ ID NO: 129 - DNA, 366 bp, synthetic construct
  misc_feature 1..366: note = Synthetic
  source 1..366: mol_type = other DNA
gaggtgcagctggtggagtctgggggaggcttggtacagcctggggggtccctaagactctcctgtgcagcctctggattcacctttagcagttatgccttgacctgggtccgccaggctccagggaaggggctggagtgggtctcttttattagtggtagtggtggtaggccattctacgcagactccgtgaagggccggttcaccatctccagagacaattccaagaacatgctgtatctgcaaatgaacagcctgagagccgaggacacggccatatattactgtgcgaagtccctgtataccaccagctggtacggggggttcgactcctggggccagggaaccctggtcaccgtctcctca

SEQ ID NO: 130 - protein, 122 aa, synthetic construct
  REGION 1..122: note = Synthetic
EVQLVESGGGLVQPGGSLRLSCAASGFTFSSYALTWVRQAPGKGLEWVSFISGSGGRPFYADSVKGRFTISRDNSKNMLYLQMNSLRAEDTAIYYCAKSLYTTSWYGGFDSWGQGTLVTVSS

SEQ ID NO: 131 - DNA, 24 bp, synthetic construct
  misc_feature 1..24: note = Synthetic
  source 1..24: mol_type = other DNA
ggattcacctttagcagttatgcc

SEQ ID NO: 132 - protein, 8 aa, synthetic construct
  REGION 1..8: note = Synthetic
GFTFSSYA

SEQ ID NO: 133 - DNA, 24 bp, synthetic construct
  misc_feature 1..24: note = Synthetic
  source 1..24: mol_type = other DNA
attagtggtagtggtggtaggcca

SEQ ID NO: 134 - protein, 8 aa, synthetic construct
  REGION 1..8: note = Synthetic
ISGSGGRP

SEQ ID NO: 135 - DNA, 45 bp, synthetic construct
  misc_feature 1..45: note = Synthetic
  source 1..45: mol_type = other DNA
gcgaagtccctgtataccaccagctggtacggggggttcgactcc

SEQ ID NO: 136 - protein, 15 aa, synthetic construct
  REGION 1..15: note = Synthetic
AKSLYTTSWYGGFDS

SEQ ID NO: 137 - DNA, 321 bp, synthetic construct
  misc_feature 1..321: note = Synthetic
  source 1..321: mol_type = other DNA
gacatccagatgacccagtctccatcttccgtgtctgcatctgtaggagacagagtcaccatcacttgtcgggcgagtcagggtgtcgtcagctggttagcctggtatcagcagaaaccagggaaagcccctaagctcctgatctatgctgcatccagtttgcaaagtggggtcccatcaaggttcagcggcagtggatctgggacagatttcactctcaccatcagcagcctgcagcctgaagattttgcaacttattattgtcaacagtctaacagtttccctttcactctcggccctgggaccaaagtggatatcaaa

SEQ ID NO: 138 - protein, 107 aa, synthetic construct
  REGION 1..107: note = Synthetic
DIQMTQSPSSVSASVGDRVTITCRASQGVVSWLAWYQQKPGKAPKLLIYAASSLQSGVPSRFSGSGSGTDFTLTISSLQPEDFATYYCQQSNSFPFTLGPGTKVDIK

SEQ ID NO: 139 - DNA, 18 bp, synthetic construct
  misc_feature 1..18: note = Synthetic
  source 1..18: mol_type = other DNA
cagggtgtcgtcagctgg

SEQ ID NO: 140 - protein, 6 aa, synthetic construct
  REGION 1..6: note = Synthetic
QGVVSW

SEQ ID NO: 141-142 - skipped (2 entries)

SEQ ID NO: 143 - DNA, 24 bp, synthetic construct
  misc_feature 1..24: note = Synthetic
  source 1..24: mol_type = other DNA
caacagtctaacagtttccctttc

SEQ ID NO: 144 - protein, 8 aa, synthetic construct
  REGION 1..8: note = Synthetic
QQSNSFPF

SEQ ID NO: 145 - DNA, 366 bp, synthetic construct
  misc_feature 1..366: note = Synthetic
  source 1..366: mol_type = other DNA
caggtgcagctggtgcagtctggggctgaagtgaagaagcctggggcctcagtgaaggtctcctgcaaggcttctggatacaccttcaccggccactatatgtactggatgcgacaggcccctggacaagggcttgagtggatgggatggatcaaccctaacagtggtggcacaaactatgcacagaagtttcaggacagggtcaccatgaccagggacacgtccatcagcacagcctacatggagctgagcaggctgagatctgacgacacggccgtgtattactgtgcgagagggagatatggcagtagctggtacggggggtttgagtactggggccagggaaccctggtcaccgtctcctca

SEQ ID NO: 146 - protein, 122 aa, synthetic construct
  REGION 1..122: note = Synthetic
QVQLVQSGAEVKKPGASVKVSCKASGYTFTGHYMYWMRQAPGQGLEWMGWINPNSGGTNYAQKFQDRVTMTRDTSISTAYMELSRLRSDDTAVYYCARGRYGSSWYGGFEYWGQGTLVTVSS

SEQ ID NO: 147 - DNA, 24 bp, synthetic construct
  misc_feature 1..24: note = Synthetic
  source 1..24: mol_type = other DNA
ggatacaccttcaccggccactat

SEQ ID NO: 148 - protein, 8 aa, synthetic construct
  REGION 1..8: note = Synthetic
GYTFTGHY

SEQ ID NO: 149 - DNA, 24 bp, synthetic construct
  misc_feature 1..24: note = Synthetic
  source 1..24: mol_type = other DNA
atcaaccctaacagtggtggcaca

SEQ ID NO: 150 - protein, 8 aa, synthetic construct
  REGION 1..8: note = Synthetic
INPNSGGT

SEQ ID NO: 151 - DNA, 45 bp, synthetic construct
  misc_feature 1..45: note = Synthetic
  source 1..45: mol_type = other DNA
gcgagagggagatatggcagtagctggtacggggggtttgagtac

SEQ ID NO: 152 - protein, 15 aa, synthetic construct
  REGION 1..15: note = Synthetic
ARGRYGSSWYGGFEY

SEQ ID NO: 153 - DNA, 321 bp, synthetic construct
  misc_feature 1..321: note = Synthetic
  source 1..321: mol_type = other DNA
gacatccagatgacccagtctccatcttccgtgtctgcatctgttggagacagagtcaccatcacttgtcgggcgagtcagggtattaccagctggttagcctggtatcagcagaaaccagggaaagcccctaacctcctgatctatgctgcagccagtttacaaagtggggtcccatcaaggttcagcggcagtggatctgggacggatttcactctcaccatcagcagcctgcagcctgaagactttacaacttactattgtcaacaggcttacagtctccctctcactttcggcggagggaccaaggtggagatcaaa

SEQ ID NO: 154 - protein, 107 aa, synthetic construct
  REGION 1..107: note = Synthetic
DIQMTQSPSSVSASVGDRVTITCRASQGITSWLAWYQQKPGKAPNLLIYAAASLQSGVPSRFSGSGSGTDFTLTISSLQPEDFTTYYCQQAYSLPLTFGGGTKVEIK

SEQ ID NO: 155 - DNA, 18 bp, synthetic construct
  misc_feature 1..18: note = Synthetic
  source 1..18: mol_type = other DNA
cagggtattaccagctgg

SEQ ID NO: 156 - protein, 6 aa, synthetic construct
  REGION 1..6: note = Synthetic
QGITSW

SEQ ID NO: 157-158 - skipped (2 entries)

SEQ ID NO: 159 - DNA, 27 bp, synthetic construct
  misc_feature 1..27: note = Synthetic
  source 1..27: mol_type = other DNA
caacaggcttacagtctccctctcact

SEQ ID NO: 160 - protein, 9 aa, synthetic construct
  REGION 1..9: note = Synthetic
QQAYSLPLT

SEQ ID NO: 161 - DNA, 366 bp, synthetic construct
  misc_feature 1..366: note = Synthetic
  source 1..366: mol_type = other DNA
caggtgcagctggtggagtctgggggaggcgtggtccagcctgggaggtccctgagactctcctgtgcagcctctggattcaccttcagtagctatggcttgcactgggtccgccagtctccaggcaaggggctggaatgggtggcacttatatcatatgacggaagtaataaatactatgcagactccgtgaagggccgattcaccatctccagagacaattccaagaacacgctgtatctgcaaatgaacagcctgagacctgaggacacggctggatatttctgtgcgaaatccctatatacaaccagctggtacgggggctttgactattggggccagggaaccctggtcaccgtctcctca

SEQ ID NO: 162 - protein, 122 aa, synthetic construct
  REGION 1..122: note = Synthetic
QVQLVESGGGVVQPGRSLRLSCAASGFTFSSYGLHWVRQSPGKGLEWVALISYDGSNKYYADSVKGRFTISRDNSKNTLYLQMNSLRPEDTAGYFCAKSLYTTSWYGGFDYWGQGTLVTVSS

SEQ ID NO: 163 - DNA, 24 bp, synthetic construct
  misc_feature 1..24: note = Synthetic
  source 1..24: mol_type = other DNA
ggattcaccttcagtagctatggc

SEQ ID NO: 164 - protein, 8 aa, synthetic construct
  REGION 1..8: note = Synthetic
GFTFSSYG

SEQ ID NO: 165 - DNA, 24 bp, synthetic construct
  misc_feature 1..24: note = Synthetic
  source 1..24: mol_type = other DNA
atatcatatgacggaagtaataaa

SEQ ID NO: 166 - protein, 8 aa, synthetic construct
  REGION 1..8: note = Synthetic
ISYDGSNK

SEQ ID NO: 167 - DNA, 45 bp, synthetic construct
  misc_feature 1..45: note = Synthetic
  source 1..45: mol_type = other DNA
gcgaaatccctatatacaaccagctggtacgggggctttgactat

SEQ ID NO: 168 - protein, 15 aa, synthetic construct
  REGION 1..15: note = Synthetic
AKSLYTTSWYGGFDY

SEQ ID NO: 169 - DNA, 321 bp, synthetic construct
  misc_feature 1..321: note = Synthetic
  source 1..321: mol_type = other DNA
gacatccagatgacccagtctccatcttccgtgtctgcatctgtaggagacagagtcaccatcacttgtcgggcgagtcagggtattagaagctggttagcctggtatcagcaaaaaccagggaaagcccctaacctcctgatctatgctgcgtccagtttgcaaagtggggtcccatcaaggttcagcggcagtggatctgggacagatttcactctcaccatcagcagcctgcagcctgaagattttgcaacttactattgtcaacaggctaacagtttccctcccactttcggccctgggaccaaagtggatatcaaa

SEQ ID NO: 170 - protein, 107 aa, synthetic construct
  REGION 1..107: note = Synthetic
DIQMTQSPSSVSASVGDRVTITCRASQGIRSWLAWYQQKPGKAPNLLIYAASSLQSGVPSRFSGSGSGTDFTLTISSLQPEDFATYYCQQANSFPPTFGPGTKVDIK

SEQ ID NO: 171 - DNA, 18 bp, synthetic construct
  misc_feature 1..18: note = Synthetic
  source 1..18: mol_type = other DNA
cagggtattagaagctgg

SEQ ID NO: 172 - protein, 6 aa, synthetic construct
  REGION 1..6: note = Synthetic
QGIRSW

SEQ ID NO: 173-174 - skipped (2 entries)

SEQ ID NO: 175 - DNA, 27 bp, synthetic construct
  misc_feature 1..27: note = Synthetic
  source 1..27: mol_type = other DNA
caacaggctaacagtttccctcccact

SEQ ID NO: 176 - protein, 9 aa, synthetic construct
  REGION 1..9: note = Synthetic
QQANSFPPT

SEQ ID NO: 177 - DNA, 366 bp, synthetic construct
  misc_feature 1..366: note = Synthetic
  source 1..366: mol_type = other DNA
gaggtgcagctggtggagtctgggggaggcttggtacagcctggggggtccctgagactctcctgtgcagcctctgggttcaccttcagcaactatgccatgacctgggtccgccaggctccagggaaggggctggagtgggtctcaactatcagtggcagtggtgataacacatactacgcagactccgtgcagggccggttcaccatctccagaggccattccaagaacacgctgtatctgcaaatgaacagcctgagagccgaggacacggccgtatattactgtgcgaaacctacgtatagcagaagctggtacggtgcttttgatttctggggccaagggacaatggtcaccgtctcttca

SEQ ID NO: 178 - protein, 122 aa, synthetic construct
  REGION 1..122: note = Synthetic
EVQLVESGGGLVQPGGSLRLSCAASGFTFSNYAMTWVRQAPGKGLEWVSTISGSGDNTYYADSVQGRFTISRGHSKNTLYLQMNSLRAEDTAVYYCAKPTYSRSWYGAFDFWGQGTMVTVSS

SEQ ID NO: 179 - DNA, 24 bp, synthetic construct
  misc_feature 1..24: note = Synthetic
  source 1..24: mol_type = other DNA
gggttcaccttcagcaactatgcc

SEQ ID NO: 180 - protein, 8 aa, synthetic construct
  REGION 1..8: note = Synthetic
GFTFSNYA

SEQ ID NO: 181 - DNA, 24 bp, synthetic construct
  misc_feature 1..24: note = Synthetic
  source 1..24: mol_type = other DNA
atcagtggcagtggtgataacaca

SEQ ID NO: 182 - protein, 8 aa, synthetic construct
  REGION 1..8: note = Synthetic
ISGSGDNT

SEQ ID NO: 183 - DNA, 45 bp, synthetic construct
  misc_feature 1..45: note = Synthetic
  source 1..45: mol_type = other DNA
gcgaaacctacgtatagcagaagctggtacggtgcttttgatttc

SEQ ID NO: 184 - protein, 15 aa, synthetic construct
  REGION 1..15: note = Synthetic
AKPTYSRSWYGAFDF

SEQ ID NO: 185 - DNA, 321 bp, synthetic construct
  misc_feature 1..321: note = Synthetic
  source 1..321: mol_type = other DNA
gacatccagatgacccagtctccatcctccgtgtctgcatctgtaggagacagagtcaccatcacttgtcgggcgagtcagggtattagcagctggttagcctggtatcagcagaaaccggggaaagcccctcaactcctgatctatgctgcatccagattgcaaagtggggtcccatcaaggttctggggcagtggatctgggacagatttcactctcaccatcagcagcctgcagcctgaagattttgcaacttactattgtcaacaggctaacaatttcccattcactttcggccctgggaccaaagtggatatcaaa

SEQ ID NO: 186 - protein, 107 aa, synthetic construct
  REGION 1..107: note = Synthetic
DIQMTQSPSSVSASVGDRVTITCRASQGISSWLAWYQQKPGKAPQLLIYAASRLQSGVPSRFWGSGSGTDFTLTISSLQPEDFATYYCQQANNFPFTFGPGTKVDIK

SEQ ID NO: 187 - DNA, 18 bp, synthetic construct
  misc_feature 1..18: note = Synthetic
  source 1..18: mol_type = other DNA
cagggtattagcagctgg

SEQ ID NO: 188 - protein, 6 aa, synthetic construct
  REGION 1..6: note = Synthetic
QGISSW

SEQ ID NO: 189-190 - skipped (2 entries)

SEQ ID NO: 191 - DNA, 27 bp, synthetic construct
  misc_feature 1..27: note = Synthetic
  source 1..27: mol_type = other DNA
caacaggctaacaatttcccattcact

SEQ ID NO: 192 - protein, 9 aa, synthetic construct
  REGION 1..9: note = Synthetic
QQANNFPFT

SEQ ID NO: 193 - DNA, 366 bp, synthetic construct
  misc_feature 1..366: note = Synthetic
  source 1..366: mol_type = other DNA
caggttcagctggtgcagtctggagctgaggtgaagaagcctggggcctcagtgaaggtctcctgcaaggcttctggttacacctttaccagttatggtatcagctgggtgcgacaggcccctggacaaggccttgagtggatgggatggatccgcgcttacaatggttacacaaactatgcacagaagtttcagggcagagtcaccatgaccacagacacatccacgaacaccgcctacatggagctgaggaccctgaattctgacgatacggccgtttattactgtgcgagagatcgatatagtgggagcttccacggtaactttgactactggggccagggaaccctggtcaccgtctcctca

SEQ ID NO: 194 - protein, 122 aa, synthetic construct
  REGION 1..122: note = Synthetic
QVQLVQSGAEVKKPGASVKVSCKASGYTFTSYGISWVRQAPGQGLEWMGWIRAYNGYTNYAQKFQGRVTMTTDTSTNTAYMELRTLNSDDTAVYYCARDRYSGSFHGNFDYWGQGTLVTVSS

SEQ ID NO: 195 - DNA, 24 bp, synthetic construct
  misc_feature 1..24: note = Synthetic
  source 1..24: mol_type = other DNA
ggttacacctttaccagttatggt

SEQ ID NO: 196 - protein, 8 aa, synthetic construct
  REGION 1..8: note = Synthetic
GYTFTSYG

SEQ ID NO: 197 - DNA, 24 bp, synthetic construct
  misc_feature 1..24: note = Synthetic
  source 1..24: mol_type = other DNA
atccgcgcttacaatggttacaca

SEQ ID NO: 198 - protein, 8 aa, synthetic construct
  REGION 1..8: note = Synthetic
IRAYNGYT

SEQ ID NO: 199 - DNA, 45 bp, synthetic construct
  misc_feature 1..45: note = Synthetic
  source 1..45: mol_type = other DNA
gcgagagatcgatatagtgggagcttccacggtaactttgactac

SEQ ID NO: 200 - protein, 15 aa, synthetic construct
  REGION 1..15: note = Synthetic
ARDRYSGSFHGNFDY

SEQ ID NO: 201 - DNA, 321 bp, synthetic construct
  misc_feature 1..321: note = Synthetic
  source 1..321: mol_type = other DNA
gacatccagatgacccagtctccatcttccgtgtctgcgtctgtaggagacagagtgaccatcacttgtcgggcgagtcagggtattttcagctggttagcctggtatcagcagaaaccagggaaagcccctaaggtcctaatctatgctgcatccaatttggaaagtggggtcccatcaaggttcagcggcagtggatctgggacagatttcactctcaccatcagcagcctgcagcctgaagattttgcaacttactattgtcaacaggctaacagtttaccgctcactttcggcggagggaccaaggtggagatcaaa

SEQ ID NO: 202 - protein, 107 aa, synthetic construct
  REGION 1..107: note = Synthetic
DIQMTQSPSSVSASVGDRVTITCRASQGIFSWLAWYQQKPGKAPKVLIYAASNLESGVPSRFSGSGSGTDFTLTISSLQPEDFATYYCQQANSLPLTFGGGTKVEIK

SEQ ID NO: 203 - DNA, 18 bp, synthetic construct
  misc_feature 1..18: note = Synthetic
  source 1..18: mol_type = other DNA
cagggtattttcagctgg

SEQ ID NO: 204 - protein, 6 aa, synthetic construct
  REGION 1..6: note = Synthetic
QGIFSW

SEQ ID NO: 205-206 - skipped (2 entries)

SEQ ID NO: 207 - DNA, 27 bp, synthetic construct
  misc_feature 1..27: note = Synthetic
  source 1..27: mol_type = other DNA
caacaggctaacagtttaccgctcact

SEQ ID NO: 208 - protein, 9 aa, synthetic construct
  REGION 1..9: note = Synthetic
QQANSLPLT

SEQ ID NO: 209 - DNA, 366 bp, synthetic construct
  misc_feature 1..366: note = Synthetic
  source 1..366: mol_type = other DNA
gaggtgcagctggtggagtctgggggaggcttggtccagcctggggggtccctgagactctcctgtgcagcctctggattcaccttcagtacctattctatgcactgggtccgccaggctccagggaagggactggaatatgtttcaactattaataataatggggataccacatattatgcagactctgtgaagggcagattcaccatctccagagacaattccaagaacacgctgtatcttcaactgggcagcctgagacctgaggacatggctgtgtattactgtgcgagacagacgtataccagcagctggtacggggggttcgactcctggggccagggaaccctggtcaccgtctcctca

SEQ ID NO: 210 - protein, 122 aa, synthetic construct
  REGION 1..122: note = Synthetic
EVQLVESGGGLVQPGGSLRLSCAASGFTFSTYSMHWVRQAPGKGLEYVSTINNNGDTTYYADSVKGRFTISRDNSKNTLYLQLGSLRPEDMAVYYCARQTYTSSWYGGFDSWGQGTLVTVSS

SEQ ID NO: 211 - DNA, 24 bp, synthetic construct
  misc_feature 1..24: note = Synthetic
  source 1..24: mol_type = other DNA
ggattcaccttcagtacctattct

SEQ ID NO: 212 - protein, 8 aa, synthetic construct
  REGION 1..8: note = Synthetic
GFTFSTYS

SEQ ID NO: 213 - DNA, 24 bp, synthetic construct
  misc_feature 1..24: note = Synthetic
  source 1..24: mol_type = other DNA
attaataataatggggataccaca

SEQ ID NO: 214 - protein, 8 aa, synthetic construct
  REGION 1..8: note = Synthetic
INNNGDTT

SEQ ID NO: 215 - DNA, 45 bp, synthetic construct
  misc_feature 1..45: note = Synthetic
  source 1..45: mol_type = other DNA
gcgagacagacgtataccagcagctggtacggggggttcgactcc

SEQ ID NO: 216 - protein, 15 aa, synthetic construct
  REGION 1..15: note = Synthetic
ARQTYTSSWYGGFDS

SEQ ID NO: 217 - DNA, 321 bp, synthetic construct
  misc_feature 1..321: note = Synthetic
  source 1..321: mol_type = other DNA
gacatccagatgacccagtctccatcttccgtgtctgcatctgtaggcgacagagtcaccatcacttgtcgggcgagtcagggtattaccagctggttagcctggtatcagcagaaaccagggaaagcccctaaactcctgatctatgctgcatccaatttgcaaagtggggtcccatcaaggttcagcggcagtggatctgggacagatttcactctcaccatcaccagcctgcagcctgaggattttgcaacttactattgtcaacaggctaacagtctcccattcactttcggccctgggaccaaagtggatatcaaa

SEQ ID NO: 218 - protein, 107 aa, synthetic construct
  REGION 1..107: note = Synthetic
DIQMTQSPSSVSASVGDRVTITCRASQGITSWLAWYQQKPGKAPKLLIYAASNLQSGVPSRFSGSGSGTDFTLTITSLQPEDFATYYCQQANSLPFTFGPGTKVDIK

SEQ ID NO: 219 - DNA, 18 bp, synthetic construct
  misc_feature 1..18: note = Synthetic
  source 1..18: mol_type = other DNA
cagggtattaccagctgg

SEQ ID NO: 220 - protein, 6 aa, synthetic construct
  REGION 1..6: note = Synthetic
QGITSW

SEQ ID NO: 221-222 - skipped (2 entries)

SEQ ID NO: 223 - DNA, 27 bp, synthetic construct
  misc_feature 1..27: note = Synthetic
  source 1..27: mol_type = other DNA
caacaggctaacagtctcccattcact

SEQ ID NO: 224 - protein, 9 aa, synthetic construct
  REGION 1..9: note = Synthetic
QQANSLPFT

SEQ ID NO: 225 - DNA, 366 bp, synthetic construct
  misc_feature 1..366: note = Synthetic
  source 1..366: mol_type = other DNA
gaggtgcagctggtggagtctgggggaggcttggtacagcctggggggtccctgagactctcctgtgcagcctctggattcacccttagcagctatgccatgagctgggtccgccaggctccagggaaggggctggagtgggtctcagctattagtggtagtggtggcagcacatactacgcagactccgtgaagggccggttcaccatctccagagacaattccaagaactcgctgtatctgcaattgaacagcctgagagccgaggacacggccgtatattactgtgcgaagacgctgtatactaccagctggtacgggggcttccagcactggggccagggcaccctggtcactgtctcctca

SEQ ID NO: 226 - protein, 122 aa, synthetic construct
  REGION 1..122: note = Synthetic
EVQLVESGGGLVQPGGSLRLSCAASGFTLSSYAMSWVRQAPGKGLEWVSAISGSGGSTYYADSVKGRFTISRDNSKNSLYLQLNSLRAEDTAVYYCAKTLYTTSWYGGFQHWGQGTLVTVSS

SEQ ID NO: 227 - DNA, 24 bp, synthetic construct
  misc_feature 1..24: note = Synthetic
  source 1..24: mol_type = other DNA
ggattcacccttagcagctatgcc

SEQ ID NO: 228 - protein, 8 aa, synthetic construct
  REGION 1..8: note = Synthetic
GFTLSSYA

SEQ ID NO: 229 - DNA, 24 bp, synthetic construct
  misc_feature 1..24: note = Synthetic
  source 1..24: mol_type = other DNA
attagtggtagtggtggcagcaca

SEQ ID NO: 230 - protein, 8 aa, synthetic construct
  REGION 1..8: note = Synthetic
ISGSGGST

SEQ ID NO: 231 - DNA, 45 bp, synthetic construct
  misc_feature 1..45: note = Synthetic
  source 1..45: mol_type = other DNA
gcgaagacgctgtatactaccagctggtacgggggcttccagcac

SEQ ID NO: 232 - protein, 15 aa, synthetic construct
  REGION 1..15: note = Synthetic
AKTLYTTSWYGGFQH

SEQ ID NO: 233 - DNA, 321 bp, synthetic construct
  misc_feature 1..321: note = Synthetic
  source 1..321: mol_type = other DNA
gacatccagatgacccagtctccatcttccgtgtctgcatctataggagacagagtcaccatcacttgtcgggcgagtcagggaatcagcagttggttagcctggtatcagcagaaaccagggaaagtccctaagctcctgatctatgctgcgtcctctttgcaaagtgggttcccatcaaggttcagcggcagtggatctgggacagatttcactctcaccatcagtagcctgcagcccgaagattttgcaacttactattgtcaacagactcacagtttcccgtggacggtcggccaagggaccaaggtggaaatcaaa

SEQ ID NO: 234 - protein, 107 aa, synthetic construct
  REGION 1..107: note = Synthetic
DIQMTQSPSSVSASIGDRVTITCRASQGISSWLAWYQQKPGKVPKLLIYAASSLQSGFPSRFSGSGSGTDFTLTISSLQPEDFATYYCQQTHSFPWTVGQGTKVEIK

SEQ ID NO: 235 - DNA, 18 bp, synthetic construct
  misc_feature 1..18: note = Synthetic
  source 1..18: mol_type = other DNA
cagggaatcagcagttgg

SEQ ID NO: 236 - protein, 6 aa, synthetic construct
  REGION 1..6: note = Synthetic
QGISSW

SEQ ID NO: 237-238 - skipped (2 entries)

SEQ ID NO: 239 - DNA, 24 bp, synthetic construct
  misc_feature 1..24: note = Synthetic
  source 1..24: mol_type = other DNA
caacagactcacagtttcccgtgg

SEQ ID NO: 240 - protein, 8 aa, synthetic construct
  REGION 1..8: note = Synthetic
QQTHSFPW

SEQ ID NO: 241 - DNA, 366 bp, synthetic construct
  misc_feature 1..366: note = Synthetic
  source 1..366: mol_type = other DNA
gaggtgcagctggtggagtctgggggaggcttggtacagcctggggggtccctgagactctcctgtgcagcctctggattcacccttaggagctatttcatgacctgggtccgccaggttccagggaaggggctggagggggtctcagctattagtggcattagtggtggcacatactacacagactccgttaagggccggttcaccatctccagagacaattccaagaacacgctgtttctgcaaatgaacagcctgagagccgaggacacggccgtatatttctgtgcgagaacggtgtatagtagtagttactacgggggcttccagcactggggccagggcaccctggtcaccgtctcctca

SEQ ID NO: 242 - protein, 122 aa, synthetic construct
  REGION 1..122: note = Synthetic
EVQLVESGGGLVQPGGSLRLSCAASGFTLRSYFMTWVRQVPGKGLEGVSAISGISGGTYYTDSVKGRFTISRDNSKNTLFLQMNSLRAEDTAVYFCARTVYSSSYYGGFQHWGQGTLVTVSS

SEQ ID NO: 243 - DNA, 24 bp, synthetic construct
  misc_feature 1..24: note = Synthetic
  source 1..24: mol_type = other DNA
ggattcacccttaggagctatttc

SEQ ID NO: 244 - protein, 8 aa, synthetic construct
  REGION 1..8: note = Synthetic
GFTLRSYF

SEQ ID NO: 245 - DNA, 24 bp, synthetic construct
  misc_feature 1..24: note = Synthetic
  source 1..24: mol_type = other DNA
attagtggcattagtggtggcaca

SEQ ID NO: 246 - protein, 8 aa, synthetic construct
  REGION 1..8: note = Synthetic
ISGISGGT

SEQ ID NO: 247 - DNA, 45 bp, synthetic construct
  misc_feature 1..45: note = Synthetic
  source 1..45: mol_type = other DNA
gcgagaacggtgtatagtagtagttactacgggggcttccagcac

SEQ ID NO: 248 - protein, 15 aa, synthetic construct
  REGION 1..15: note = Synthetic
ARTVYSSSYYGGFQH

SEQ ID NO: 249 - DNA, 321 bp, synthetic construct
  misc_feature 1..321: note = Synthetic
  source 1..321: mol_type = other DNA
gacatccagatgacccagtctccatcttccgtgtctgtatctgtaggagacagagtcaccatcacttgtcgggcgagtcagggtattagcagttggttagcctggtatcagcagaaaccagggaaagcccctaagctcctgatctatgttgcatccagtttacaaagtggggtcccatcaaggttcagcggcagtggatctgggacagatttcactctcaccatcagcagcctgcagcctgaagattttgcaacttactattgtcaacagactaacagtttccctctcactttcggcggagggaccaaggtggagatcaaa

SEQ ID NO: 250 - protein, 107 aa, synthetic construct
  REGION 1..107: note = Synthetic
DIQMTQSPSSVSVSVGDRVTITCRASQGISSWLAWYQQKPGKAPKLLIYVASSLQSGVPSRFSGSGSGTDFTLTISSLQPEDFATYYCQQTNSFPLTFGGGTKVEIK

SEQ ID NO: 251 - DNA, 18 bp, synthetic construct
  misc_feature 1..18: note = Synthetic
  source 1..18: mol_type = other DNA
cagggtattagcagttgg

SEQ ID NO: 252 - protein, 6 aa, synthetic construct
  REGION 1..6: note = Synthetic
QGISSW

SEQ ID NO: 253-254 - skipped (2 entries)

SEQ ID NO: 255 - DNA, 27 bp, synthetic construct
  misc_feature 1..27: note = Synthetic
  source 1..27: mol_type = other DNA
caacagactaacagtttccctctcact

SEQ ID NO: 256 - protein, 9 aa, synthetic construct
  REGION 1..9: note = Synthetic
QQTNSFPLT

SEQ ID NO: 257 - DNA, 366 bp, synthetic construct
  misc_feature 1..366: note = Synthetic
  source 1..366: mol_type = other DNA
gaggtgcagctggtggagtctgggggaggcttggtacagcctggggggtccctgagactctcctgtgcagcctctggattcacccttaggagttatgtcatgtactgggtccgccagggtccagggaaggggctggagggggtctcaggtattagtggcagtagtggtggcacatactacacagactccgtgaagggccggttcaccatctccagagacaattccaagaacacgctgtttctgcaaatgaacagcctgagagccgaggacacggccgtatatttctgtgcgagatcggtgtatagtaccacctggtacgggggcttccagcactggggccagggcaccctggtcaccgtctcctca

SEQ ID NO: 258 - protein, 122 aa, synthetic construct
  REGION 1..122: note = Synthetic
EVQLVESGGGLVQPGGSLRLSCAASGFTLRSYVMYWVRQGPGKGLEGVSGISGSSGGTYYTDSVKGRFTISRDNSKNTLFLQMNSLRAEDTAVYFCARSVYSTTWYGGFQHWGQGTLVTVSS

SEQ ID NO: 259 - DNA, 24 bp, synthetic construct
  misc_feature 1..24: note = Synthetic
  source 1..24: mol_type = other DNA
ggattcacccttaggagttatgtc

SEQ ID NO: 260 - protein, 8 aa, synthetic construct
  REGION 1..8: note = Synthetic
GFTLRSYV

SEQ ID NO: 261 - DNA, 24 bp, synthetic construct
  misc_feature 1..24: note = Synthetic
  source 1..24: mol_type = other DNA
attagtggcagtagtggtggcaca

SEQ ID NO: 262 - protein, 8 aa, synthetic construct
  REGION 1..8: note = Synthetic
ISGSSGGT

SEQ ID NO: 263 - DNA, 45 bp, synthetic construct
  misc_feature 1..45: note = Synthetic
  source 1..45: mol_type = other DNA
gcgagatcggtgtatagtaccacctggtacgggggcttccagcac

SEQ ID NO: 264 - protein, 15 aa, synthetic construct
  REGION 1..15: note = Synthetic
ARSVYSTTWYGGFQH

SEQ ID NO: 265 - DNA, 321 bp, synthetic construct
  misc_feature 1..321: note = Synthetic
  source 1..321: mol_type = other DNA
gacatccagatgacccagtctccatcttccgtgtctgtatctgtgggagacagagtcaccatcacttgtcgggcgagtcaggttattagcagttggttagcctggtatcagctgaaaccagggaaagcccctaaactcctgatctatgctgcatccagtttacaaagtggggtcccatcaaggttcagcggcagtggatctgggacagatttcactctcaccatcagcggcctgcagcctgaagattttgcagtttactattgtcaacagactaacagtttccctctcactttcggcggagggaccaaggtggagatcaaa

SEQ ID NO: 266 - protein, 107 aa, synthetic construct
  REGION 1..107: note = Synthetic
DIQMTQSPSSVSVSVGDRVTITCRASQVISSWLAWYQLKPGKAPKLLIYAASSLQSGVPSRFSGSGSGTDFTLTISGLQPEDFAVYYCQQTNSFPLTFGGGTKVEIK

SEQ ID NO: 267 - DNA, 18 bp, synthetic construct
  misc_feature 1..18: note = Synthetic
  source 1..18: mol_type = other DNA
caggttattagcagttgg

SEQ ID NO: 268 - protein, 6 aa, synthetic construct
  REGION 1..6: note = Synthetic
QVISSW

SEQ ID NO: 269-270 - skipped (2 entries)

SEQ ID NO: 271 - DNA, 27 bp, synthetic construct
  misc_feature 1..27: note = Synthetic
  source 1..27: mol_type = other DNA
caacagactaacagtttccctctcact

SEQ ID NO: 272 - protein, 9 aa, synthetic construct
  REGION 1..9: note = Synthetic
QQTNSFPLT

SEQ ID NO: 273 - DNA, 366 bp, synthetic construct
  misc_feature 1..366: note = Synthetic
  source 1..366: mol_type = other DNA
gaggtgcagctggtggagtctgggggaaacttggaacagcctggggggtcccttagactctcctgtacagcctctggattcacctttagcagatctgccatgaactgggtccgccgggctccagggaaggggctggagtgggtctcaggaattagtggtagtggtggtcgaacatactacgcagactccgtgaagggccggttcaccatctccagagacaattccaagaatacgctatatctgcaaatgaacagcctgagcgccgaggacacggccgcatattactgtgcgaaagattcgtatactaccagttggtacggaggtatggacgtctggggccacgggaccacggtcaccgtctcctca

SEQ ID NO: 274 - protein, 122 aa, synthetic construct
  REGION 1..122: note = Synthetic
EVQLVESGGNLEQPGGSLRLSCTASGFTFSRSAMNWVRRAPGKGLEWVSGISGSGGRTYYADSVKGRFTISRDNSKNTLYLQMNSLSAEDTAAYYCAKDSYTTSWYGGMDVWGHGTTVTVSS

SEQ ID NO: 275 - DNA, 24 bp, synthetic construct
  misc_feature 1..24: note = Synthetic
  source 1..24: mol_type = other DNA
ggattcacctttagcagatctgcc

SEQ ID NO: 276 - protein, 8 aa, synthetic construct
  REGION 1..8: note = Synthetic
GFTFSRSA

SEQ ID NO: 277 - DNA, 24 bp, synthetic construct
  misc_feature 1..24: note = Synthetic
  source 1..24: mol_type = other DNA
attagtggtagtggtggtcgaaca

SEQ ID NO: 278 - protein, 8 aa, synthetic construct
  REGION 1..8: note = Synthetic
ISGSGGRT

SEQ ID NO: 279 - DNA, 45 bp, synthetic construct
  misc_feature 1..45: note = Synthetic
  source 1..45: mol_type = other DNA
gcgaaagattcgtatactaccagttggtacggaggtatggacgtc

SEQ ID NO: 280 - protein, 15 aa, synthetic construct
  REGION 1..15: note = Synthetic
AKDSYTTSWYGGMDV

SEQ ID NO: 281 - DNA, 321 bp, synthetic construct
  misc_feature 1..321: note = Synthetic
  source 1..321: mol_type = other DNA
gacatccagatgacccagtctccatcttccgtgtctgcatctgtaggagacagagtcaccatcacttgtcgggcgagtcagggtattttcagctggttagcctggtatcagcagaaaccaggaaaagcccctaagctcctgatctatgctgcttccagtttacaaagtggggtcccatcaagattcagcggcagtggatctgggacagatttcactctcaccatcagcagcctgcagcctgaggattttgcaatttactattgtcaacaggctaacagtgtcccgatcaccttcggccaagggacacgactggagattaaa

SEQ ID NO: 282 - protein, 107 aa, synthetic construct
  REGION 1..107: note = Synthetic
DIQMTQSPSSVSASVGDRVTITCRASQGIFSWLAWYQQKPGKAPKLLIYAASSLQSGVPSRFSGSGSGTDFTLTISSLQPEDFAIYYCQQANSVPITFGQGTRLEIK

SEQ ID NO: 283 - DNA, 18 bp, synthetic construct
  misc_feature 1..18: note = Synthetic
  source 1..18: mol_type = other DNA
cagggtattttcagctgg

SEQ ID NO: 284 - protein, 6 aa, synthetic construct
  REGION 1..6: note = Synthetic
QGIFSW

SEQ ID NO: 285-286 - skipped (2 entries)

SEQ ID NO: 287 - DNA, 27 bp, synthetic construct
  misc_feature 1..27: note = Synthetic
  source 1..27: mol_type = other DNA
caacaggctaacagtgtcccgatcacc

SEQ ID NO: 288 - protein, 9 aa, synthetic construct
  REGION 1..9: note = Synthetic
QQANSVPIT

SEQ ID NO: 289 - DNA, 366 bp, synthetic construct
  misc_feature 1..366: note = Synthetic
  source 1..366: mol_type = other DNA
gaggtgcagctggtggagtctgggggaggcttggtacagcctggggggtccctgagactctcctgttcagcctctggattcacctttagcagctatgccatgaactgggtccgccaggctccagggaaggggctggagtgggtcaccgctattagtggcagtggtggtggcacatactacgcagactccgtgaagggccggttcaccatctccagagacaattccaagaactcgctgtttctgcaattgaacagcctgagagccgaggacacggccgtgtattactgtgcgaaacaaacgtataccagcagctggtacggtggctttgatatctggggccaggggacaatggtcaccgtctcttca

SEQ ID NO: 290 - protein, 122 aa, synthetic construct
  REGION 1..122: note = Synthetic
EVQLVESGGGLVQPGGSLRLSCSASGFTFSSYAMNWVRQAPGKGLEWVTAISGSGGGTYYADSVKGRFTISRDNSKNSLFLQLNSLRAEDTAVYYCAKQTYTSSWYGGFDIWGQGTMVTVSS

SEQ ID NO: 291 - DNA, 24 bp, synthetic construct
  misc_feature 1..24: note = Synthetic
  source 1..24: mol_type = other DNA
ggattcacctttagcagctatgcc

SEQ ID NO: 292 - protein, 8 aa, synthetic construct
  REGION 1..8: note = Synthetic
GFTFSSYA

SEQ ID NO: 293 - DNA, 24 bp, synthetic construct
  misc_feature 1..24: note = Synthetic
  source 1..24: mol_type = other DNA
attagtggcagtggtggtggcaca

SEQ ID NO: 294 - protein, 8 aa, synthetic construct
  REGION 1..8: note = Synthetic
ISGSGGGT

SEQ ID NO: 295 - DNA, 45 bp, synthetic construct
  misc_feature 1..45: note = Synthetic
  source 1..45: mol_type = other DNA
gcgaaacaaacgtataccagcagctggtacggtggctttgatatc

SEQ ID NO: 296 - protein, 15 aa, synthetic construct
  REGION 1..15: note = Synthetic
AKQTYTSSWYGGFDI

SEQ ID NO: 297 - DNA, 321 bp, synthetic construct
  misc_feature 1..321: note = Synthetic
  source 1..321: mol_type = other DNA
gacatccagatgacccagtcgccatcttccgtgtccgcgtctgtaggagacagagtcaccatcacttgtcgggcgagtcagggttttagttcctggttagcctggtatcagcagataccagggaaagcccccaagctcctgatctatgctgcatcaaggttgcaaagtggggtcccatccaggttccgcggcagtggatctgggacagatttcactctcaccatcagcagcctgcagcctgaggattttgcaacttactattgtcaacaggctaacagtttcccgctcactttcggcggagggaccaaggtggagatcaaa

SEQ ID NO: 298 - protein, 107 aa, synthetic construct
  REGION 1..107: note = Synthetic
DIQMTQSPSSVSASVGDRVTITCRASQGFSSWLAWYQQIPGKAPKLLIYAASRLQSGVPSRFRGSGSGTDFTLTISSLQPEDFATYYCQQANSFPLTFGGGTKVEIK

SEQ ID NO: 299 - DNA, 18 bp, synthetic construct
  misc_feature 1..18: note = Synthetic
  source 1..18: mol_type = other DNA
cagggttttagttcctgg

SEQ ID NO: 300 - protein, 6 aa, synthetic construct
  REGION 1..6: note = Synthetic
QGFSSW

SEQ ID NO: 301-302 - skipped (2 entries)

SEQ ID NO: 303 - DNA, 27 bp, synthetic construct
  misc_feature 1..27: note = Synthetic
  source 1..27: mol_type = other DNA
caacaggctaacagtttcccgctcact

SEQ ID NO: 304 - protein, 9 aa, synthetic construct
  REGION 1..9: note = Synthetic
QQANSFPLT

SEQ ID NO: 305 - protein, 167 aa, synthetic construct
  REGION 1..167: note = Synthetic
SITGISPITESLASLSTYNDQSITFALEDESYEIYVEDLKKDKKKDKVLLSYYESQHPSSESGDGVDGKMLMVTLSPTKDFWLQANNKEHSVELHKCEKPLPDQAFFVLHNRSFNCVSFECKTDPGVFIGVKDNHLALIKVDYSENLGSENILFKLSEILEHHHHHH

SEQ ID NO: 306 - protein, 167 aa, synthetic construct; identical to SEQ ID NO: 305
  REGION 1..167: note = Synthetic

SEQ ID NO: 307 - DNA, 354 bp, synthetic construct
  misc_feature 1..354: note = Synthetic
  source 1..354: mol_type = other DNA
caggtcaccttgaaggagtctggtcctgtgctggtgaaacccacagagagcctcacgctgacctgctccgtctctggattctcactcagtaatgttagaatgggtgtgagctggatccgtcagtccccagggaaggccctggagtggcttgcacacattttttcgaatgacgaaaaatcctacaccacatctctgaagaccaggctcaccatctccaaggacacctccagaagccaggtggtccttaccatgaccgacatggaccctggggacacagccacatattactgtgcacggatacggaatttggcctttaattactggggccagggaaccctggtcaccgtctcctca

SEQ ID NO: 308 - protein, 118 aa, synthetic construct
  REGION 1..118: note = Synthetic
QVTLKESGPVLVKPTESLTLTCSVSGFSLSNVRMGVSWIRQSPGKALEWLAHIFSNDEKSYTTSLKTRLTISKDTSRSQVVLTMTDMDPGDTATYYCARIRNLAFNYWGQGTLVTVSS

SEQ ID NO: 309 - DNA, 30 bp, synthetic construct
  misc_feature 1..30: note = Synthetic
  source 1..30: mol_type = other DNA
ggattctcactcagtaatgttagaatgggt

SEQ ID NO: 310 - protein, 10 aa, synthetic construct
  REGION 1..10: note = Synthetic
GFSLSNVRMG

SEQ ID NO: 311 - DNA, 21 bp, synthetic construct
  misc_feature 1..21: note = Synthetic
  source 1..21: mol_type = other DNA
attttttcgaatgacgaaaaa

SEQ ID NO: 312 - protein, 7 aa, synthetic construct
  REGION 1..7: note = Synthetic
IFSNDEK

SEQ ID NO: 313 - DNA, 30 bp, synthetic construct
  misc_feature 1..30: note = Synthetic
  source 1..30: mol_type = other DNA
gcacggatacggaatttggcctttaattac

SEQ ID NO: 314 - protein, 10 aa, synthetic construct
  REGION 1..10: note = Synthetic
ARIRNLAFNY

SEQ ID NO: 315 - DNA, 339 bp, synthetic construct
  misc_feature 1..339: note = Synthetic
  source 1..339: mol_type = other DNA
gacttcgtgatgacccagtctccagactccctggctgtgtctctgggcgagagggccaccatcaactgcaagtccagccagagtgtgttacacaggtccagcaataagaactacttagcttggtatcagcagaagccaggacagcctcctaacctgctcatttactgggcatctacccgggaatccggggtccctgaccgattcagtggcagcgggtctgggacagatttcactctcaccatcagcagcctgcaggctgaagatgtggcagtttattactgtcagcaatattatggtactctatttactttcggccctgggaccaaagtggatatcaaa

SEQ ID NO: 316 - protein, 113 aa, synthetic construct
  REGION 1..113: note = Synthetic
DFVMTQSPDSLAVSLGERATINCKSSQSVLHRSSNKNYLAWYQQKPGQPPNLLIYWASTRESGVPDRFSGSGSGTDFTLTISSLQAEDVAVYYCQQYYGTLFTFGPGTKVDIK

SEQ ID NO: 317 - DNA, 36 bp, synthetic construct
  misc_feature 1..36: note = Synthetic
  source 1..36: mol_type = other DNA
cagagtgtgttacacaggtccagcaataagaactac

SEQ ID NO: 318 - protein, 12 aa, synthetic construct
  REGION 1..12: note = Synthetic
QSVLHRSSNKNY

SEQ ID NO: 319-320 - skipped (2 entries)

SEQ ID NO: 321 - DNA, 27 bp, synthetic construct
  misc_feature 1..27: note = Synthetic
  source 1..27: mol_type = other DNA
cagcaatattatggtactctatttact

SEQ ID NO: 322 - protein, 9 aa, synthetic construct
  REGION 1..9: note = Synthetic
QQYYGTLFT

SEQ ID NO: 323 - protein, 338 aa, synthetic construct
  REGION 1..338: note = synthetic Amino acids 1-310: Human ST2 (K19-S328 of accession number NP_057316.3) Amino acids 311-338: Myc-Myc-hexahistidine tag
KFSKQSWGLENEALIVRCPRQGKPSYTVDWYYSQTNKSIPTQERNRVFASGQLLKFLPAAVADSGIYTCIVRSPTFNRTGYANVTIYKKQSDCNVPDYLMYSTVSGSEKNSKIYCPTIDLYNWTAPLEWFKNCQALQGSRYRAHKSFLVIDNVMTEDAGDYTCKFIHNENGANYSVTATRSFTVKDEQGFSLFPVIGAPAQNEIKEVEIGKNANLTCSACFGKGTQFLAAVLWQLNGTKITDFGEPRIQQEEGQNQSFSNGLACLDMVLRIADVKEEDLLLQYDCLALNLHGLRRHTVRLSRKNPIDHHSEQKLISEEDLGGEQKLISEEDLHHHHHH